European Patent Specification EP 3 967 766 B1, published April 10, 2024. Title: PRIMER PROBE COMBINATION, KIT, DETECTION METHOD AND APPLICATION FOR DETECTING SEPARATE CANDIDA TYPES. Applicant: DYNAMIKER BIOTECHNOLOGY (TIANJIN) CO., LTD. The sequence listing filed with the application follows.

SEQUENCE LISTING (29 sequences)

SEQ ID NO: 1 - DNA, 18 bp, Synthetic sequence
tgtttgagcgtcgtttct

SEQ ID NO: 2 - DNA, 18 bp, Synthetic sequence
aagttcagcgggtagtcc

SEQ ID NO: 3 - DNA, 20 bp, Synthetic sequence
gcctgtttgagcgtcgtttc

SEQ ID NO: 4 - DNA, 20 bp, Synthetic sequence
cgccttaccactaccgtctt

SEQ ID NO: 5 - DNA, 19 bp, Synthetic sequence
ctgtttgagcgtcgtttct

SEQ ID NO: 6 - DNA, 19 bp, Synthetic sequence
taagttcagcgggtagtcc

SEQ ID NO: 7 - DNA, 20 bp, Synthetic sequence
agtactacactgcgtgagcg

SEQ ID NO: 8 - DNA, 20 bp, Synthetic sequence
tgcgagaaccaagagatccg

SEQ ID NO: 9 - DNA, 20 bp, Synthetic sequence
aacgcagcgaaatgcgatac

SEQ ID NO: 10 - DNA, 20 bp, Synthetic sequence
ggaataccagagggcgcaat

SEQ ID NO: 11 - DNA, 25 bp, Synthetic sequence
atcactgtacttgttcgctatcggt

SEQ ID NO: 12 - DNA, 25 bp, Synthetic sequence
tttccactcattggtacaaactcca

SEQ ID NO: 13 - DNA, 20 bp, Synthetic sequence
acgcacactcccaggtcttt

SEQ ID NO: 14 - DNA, 27 bp, Synthetic sequence
tcctccgtctatgctccgttacctgtt

SEQ ID NO: 15 - DNA, 24 bp, Synthetic sequence
aaacgcttattttgctagtggcca

SEQ ID NO: 16 - DNA, 25 bp, Synthetic sequence
tagtgacatgaacaagcgataacca

SEQ ID NO: 17 - DNA, 25 bp, Synthetic sequence
aaaggcgagaaaccaagttagaggt

SEQ ID NO: 18 - DNA, 20 bp, Synthetic sequence
tgcgagtgagggaccagaaa

SEQ ID NO: 19 - DNA, 27 bp, Synthetic sequence
aggatgcacatacgagacaatggacaa

SEQ ID NO: 20 - DNA, 24 bp, Synthetic sequence
tttgcgaataaaaccatcaccggt

SEQ ID NO: 21 - DNA, 18 bp, Synthetic sequence
ctgtgaatgccatttctc

SEQ ID NO: 22 - DNA, 18 bp, Synthetic sequence
acacctcctttggaatag

SEQ ID NO: 23 - DNA, 24 bp, Synthetic sequence
cctaacctacccgccttggatatt

SEQ ID NO: 24 - DNA, 809 bp, Synthetic sequence
catgattcagccaacataacccgacccgtacaattctattacgcgtctccggcgactgactatacttgccgttcggagttagggttttactccgagagaaaattgagtcagcgatgaatccgttgacaaggtgaagaagacgcagagcattaacgcgaaagaattagatctagggatttacgacgaagcatcttggcacgccaagtacaaagattcagcctacgtttacgtcggagaattaccttacgatctcacggagggtgacctcctcgccgttttctcacaatatggtgaagttgttgatttgaatcttgttcgagataaaggaactgggagatcaaaaagatttgcgtttgttgcttatgaagatcagagaagtactaatcttgctgttggataataaaagtggagcattgtggtaaatacttaaagagagaagaggaagatgaagagacgaagcagaagaagagagaagctccgtggtgtttgcagagcttttcagagaaaggagtgtactcgtggagattcttgcaaattttctcacgatgaaaatagagctgccaataccgggtggggtcacgaagatcgtagaagttccaagtgagagatcaagtaagtaaataccataatgatgtagaggataaatagggattgttcatattgatatccaagtggtaatgctctacattgaagaatggtttctaagttgtagctagaatctaatggaaaatgtgatttattgaccattagcttacacaccggtgttttgctctgtatatgtcgatcttattttcagtgttcacctttac

SEQ ID NO: 25 - DNA, 593 bp, Synthetic sequence
atatcaataagcggaggaaaagaaaccaacagggattgcctcagtagcggcgagtgaagcggcaaaagctcaaatttgaaatctggcgtctttggcgtccgagttgtaatttgaagaaggtatctttgggcccggctcttgtctatgttccttggaacaggacgtcacagagggtgagaatcccgtgcgatgagatgacccgggtctgtgtaaagttccttcgacgagtcgagttgtttgggaatgcagctctaagtgggtggtaaattccatctaaagctaaatattggcgagagaccgatagcgaacaagtacagtgatggaaagatgaaaagaactttgaaaagagagtgaaaaagtacgtgaaattgttgaaagggaagggcttgagatcagacttggtattttgcatgctgctctctcgggggcggccgctgcggtttaccgggccagcatcggtttggagcggcaggataatggcggaggaatgtggcacggcttctgctgtgtgttatagcctctgacgatactgccagcctagaccgaggactgcggtttttacctaggatgttggcataatgatcttaagtcgc

SEQ ID NO: 26 - DNA, 865 bp, Synthetic sequence
aaaagaaaccaacagggattgccttagtagcggcgagtgaagcggcaaaagctcaaatttgaaatctggctctttcagagtccgagttgtaatttgaagaaggtatctttgggtctggctcttgtctatgtttcttggaacagaacgtcacagagggtgagaatcccgtgcgatgagatgatccaggcctatgtaaagttccttcgaagagtcgagttgtttgggaatgcagctctaagtgggtggtaaattccatctaaagctaaatattggcgagagaccgatagcgaacaagtacagtgatggaaagatgaaaagaactttgaaaagagagtgaaaaagtacgtgaaattgttgaaagggaagggcttgagatcagacttggtattttgtatgttacttcttcgggggtggcctctacagtttatcgggccagcatcagtttgggcggtaggagaattgcgttggaatgtggcacggcttcggttgtgtgttatagccttcgtcgatactgccagcctagactgaggactgcggtttatacctaggatgttggcataatgatcttaagtcgcccgtcttgaaacacggaccaaggagtctaacgtctatgcgagtgtttgggtgtaaaacccgtacgcgtaatgaaagtgaacgtaggtgggggcccgtatgggtgcaccatcgaccgatcctgatgtcttcggatggatttgagtaagagcatagctgttgggacccgaaagatggtgaactatgcctgaatagggtgaagccagaggaaactctggtggaggctcgtagcggttctgacgtgcaaatcgatcgtcgaatttgggtataggggcgaaagactaatcgaccc

SEQ ID NO: 27 - DNA, 613 bp, Synthetic sequence
gcatatcaataagcggaggaaaagaaaccaacagggattgccttagtagcggcgagtgaagcggcaaaagctcaaatttgaaatctggcactttcagtgtccgagttgtaatttgaagaaggtatctttgggtctggctcttgtctatgtttcttggaacagaacgtcacagagggtgagaatcccgtgcgatgagatgtcccagacctatgtaaagttccttcgaagagtcgagttgtttgggaatgcagctctaagtgggtggtaaattccatctaaagctaaatattggcgagagaccgatagcgaacaagtacagtgatggaaagatgaaaagaactttgaaaagagagtgaaaaagtacgtgaaattgttgaaagggaagggcttgagatcagacttggtattttgtatgttactctctcgggggtggcctctacagtttaccgggccagcatcagtttgagcggtaggataagtgcaaagaaatgtggcactgcttcggtagtgtgttatagtctttgtcgatactgccagcttagactgaggactgcggcttcggcctaggatgttggcataatgatcttaagtcgcccgtcttgaaacacggacc

SEQ ID NO: 28 - DNA, 631 bp, Synthetic sequence
tttcatgcgcttgatttttcaagccaaccatcgaaagggaatccggttaaaattccggaacttggatatggattcttcacggcaacgtaactgaatgtggagacgtcggcgtgagccctgggaggagttatcttttcttcttaacagcttatcaccctggaattggtttatccggagatggggtcttatggctggaagagcgcggtaattttgccgcgtccggtgcgctcacgacggtccttgaaaatccacaggaaggaatagttttcatgccaagtcgtactcataaccgcagcaggtctccaaggttaacagcctctagttgatagaataatgtagataagggaagtcggcaaaatagatccgtaacttcgggataaggattggctctaaggatcgggtggtttgggccttgcgtagaagtggtggtgactggcggcgggctgctttcgggcggactgctgttggacgtcgctatagacacacttggtaggcatttatgtcgtccggatcacgcttaacgatcaacttagaactggtacggacaaggggaatctgactgtctaattaaaacatagcattgtgatggtcagaaagtgatgttgacacaatgtgatttctgcccagtgct

SEQ ID NO: 29 - DNA, 872 bp, Synthetic sequence
gccttagtaacggcgagtgaagcggcaaaagctcaaatttgaaatctggtacctttggtgcccgagttgtaatttggagagtaccactttgggactgtactttgcctatgttccttggaacaggacgtcatggagggtgagaatcccgtgtggcgaggtgtgtcagttctttgtaaagggtgctcgaagagtcgagttgtttgggaatgcagctctaagtgggtggtaaattccatctaaagctaaatacaggcgagagaccgatagcgaacaagtacagtgatggaaagatgaaaagaactttgaaaagagagtgaaaaagtacgtgaaattgttgaaagggaagggcatttgatcagacatggtgttttgcgccttgcctctcgtggggggactctcgcagctcactgggccagcatcggttttggcggccggaaaaaacctagggaatgtggctctgcctcggtgtagagttatagccctggggaatacggccagccgggaccgaggactgcgatttgtatctaggatgctggcataatggttatatgccgcccgtcttgaaacacggaccaaggagtctaacgtctatgcgagtgtttgggtgttaaacccgtacgcgtaatgaaagtgaacgtaggttgggcccctggggggtgcacaatcgaccgatcctgatgtcttcggatggatttgagtaagagcatagctgttgggacccgaaagatggtgaactatgcctgaatagggtgaagccagaggaaactctggtggaggctcgtagcggttctgacgtgcaaatcgatcgtcgaatttgggtataggggcgaaagactaatcgaaccatctagtagctggttcctgccgaagtt